European Patent Application EP 4 686 765 A1, published February 4, 2026. Title: METHOD FOR PROGNOSIS OF BLADDER CANCER. Applicant: Istituto Europeo di Oncologia. The sequence listing filed with the application follows.

SEQUENCE LISTING (20 sequences)

SEQ ID NO: 1 - RNA, 19 nt, synthetic construct
  source 1..19: mol_type = other RNA
cagccactgaacaagcaga

SEQ ID NO: 2 - RNA, 19 nt, synthetic construct
  source 1..19: mol_type = other RNA
agacgaacaagtcaccgac

SEQ ID NO: 3 - DNA, 36 bp, synthetic construct
  source 1..36: mol_type = other DNA
tttttctcgagacgcgtatcgattgaattggccacc

SEQ ID NO: 4 - DNA, 26 bp, synthetic construct
  source 1..26: mol_type = other DNA
ctgcaggaattcttacaacagcaggc

SEQ ID NO: 5 - DNA, 42 bp, synthetic construct
  source 1..42: mol_type = other DNA
tttttctcgagacgcgtatggagcagaagctgatctccgagg

SEQ ID NO: 6 - DNA, 22 bp, synthetic construct
  source 1..22: mol_type = other DNA
ggatatctgcagaattcaccgc

SEQ ID NO: 7 - DNA, 19 bp, synthetic construct
  source 1..19: mol_type = other DNA
gtggaagggctcatgacca

SEQ ID NO: 8 - DNA, 20 bp, synthetic construct
  source 1..20: mol_type = other DNA
ggatgcagggatgatgttct

SEQ ID NO: 9 - DNA, 19 bp, synthetic construct
  source 1..19: mol_type = other DNA
acctgtgggatgggcatct

SEQ ID NO: 10 - DNA, 20 bp, synthetic construct
  source 1..20: mol_type = other DNA
caggcggctctgcttctcta

SEQ ID NO: 11 - DNA, 19 bp, synthetic construct
  source 1..19: mol_type = other DNA
ccaatgacaacgcctcctg

SEQ ID NO: 12 - DNA, 19 bp, synthetic construct
  source 1..19: mol_type = other DNA
tggtgcagccagaaagctc

SEQ ID NO: 13 - DNA, 18 bp, synthetic construct
  source 1..18: mol_type = other DNA
aaatcccccgaaccagtc

SEQ ID NO: 14 - DNA, 21 bp, synthetic construct
  source 1..21: mol_type = other DNA
gggccggtatttcttcacact

SEQ ID NO: 15 - DNA, 21 bp, synthetic construct
  source 1..21: mol_type = other DNA
agcctcgcatcctatacaacc

SEQ ID NO: 16 - DNA, 21 bp, synthetic construct
  source 1..21: mol_type = other DNA
ttctttcacaaggcggcactc

SEQ ID NO: 17 - DNA, 21 bp, synthetic construct
  source 1..21: mol_type = other DNA
cgtggaggaaacctggatgtt

SEQ ID NO: 18 - DNA, 21 bp, synthetic construct
  source 1..21: mol_type = other DNA
gtgctgagcaacttatctcgg

SEQ ID NO: 19 - DNA, 20 bp, synthetic construct
  source 1..20: mol_type = other DNA
agcgcccgagataagttgct

SEQ ID NO: 20 - DNA, 20 bp, synthetic construct
  source 1..20: mol_type = other DNA
caccagatccatcggcgtct